European Patent Application EP 4 378 475 A1, published June 5, 2024. Title: RECOMBINANT ANTIGEN FOR INDUCING AN IMMUNE RESPONSE AGAINST THE ZIKA VIRUS. Applicant: CENTRO DE INGENIERIA GENETICA Y BIOTECNOLOGIA. Application CU 2021-0063, filed July 28, 2021. The sequence listing filed with the application follows.

SEQUENCE LISTING (11 sequences)

SEQ ID NO: 1 - DNA, 22 bp, synthetic construct
  source 1..22: mol_type = other DNA
catgatactgctgattgccccg

SEQ ID NO: 2 - DNA, 22 bp, synthetic construct
  source 1..22: mol_type = other DNA
gaagtccactgagcaccccacg

SEQ ID NO: 3 - DNA, 27 bp, synthetic construct
  source 1..27: mol_type = other DNA
atttggaaacgagagtttctggtcatg

SEQ ID NO: 4 - DNA, 24 bp, synthetic construct
  source 1..24: mol_type = other DNA
cggcatcgctcctatccaagtaca

SEQ ID NO: 5 - DNA, 25 bp, synthetic construct
  source 1..25: mol_type = other DNA
cacttaggatcccgcctgaaaatgg

SEQ ID NO: 6 - DNA, 24 bp, synthetic construct
  source 1..24: mol_type = other DNA
gttggatccgcctccaactgatcc

SEQ ID NO: 7 - DNA, 26 bp, synthetic construct
  source 1..26: mol_type = other DNA
cgagagtttctgggatccaaaaaccc

SEQ ID NO: 8 - DNA, 33 bp, synthetic construct
  source 1..33: mol_type = other DNA
actagtaagctttcatcgtctcttcttctcctt

SEQ ID NO: 9 - protein, 113 aa, synthetic construct
MGHHHHHHGSKNPKKKSGGFRIVNMLKRGVARVSPFGGLKRLPAGLLLGHGPIRMVLAILAFLRFTAIKPSLGLINRWGSVGKKEAMEIIKKFKKDLAAMLRIINARKEKKRR

SEQ ID NO: 10 - protein, 260 aa, synthetic construct
MGHHHHHHGSRLKMDKLRLKGVSYSLCTAAFTFTKIPAETLHGTVTVEVQYAGTDGPCKVPAQMAVDMQTLTPVGRLITANPVITESTENSKMMLELDPPFGDSYIVIGVGEKKITHHWYRSGSTIGKAFEATVRGAKRMAVLGDTAWDFGSVGGGSKNPKKKSGGFRIVNMLKRGVARVSPFGGLKRLPAGLLLGHGPIRMVLAILAFLRFTAIKPSLGLINRWGSVGKKEAMEIIKKFKKDLAAMLRIINARKEKKRR

SEQ ID NO: 11 - DNA, 39 bp, synthetic construct
  source 1..39: mol_type = other DNA
atcgactctcgagcgttctcgggggacgatcgtcggggg